European Patent Application EP 4 779 033 A1, published July 22, 2026. Title: 우유의 β-카제인 A1 형 유전자와 β-카제인 A2 형 유전자 검출용 조성물 및 검출 방법. Applicant: 주식회사 미코바이오메드. Application KR. The sequence listing filed with the application follows.

SEQUENCE LISTING (7 sequences)

SEQ ID NO: 1 - DNA, 21 bp, Synthetic construct
  source 1..21: mol_type = other DNA
gcccagacacagtctctagtc

SEQ ID NO: 2 - DNA, 24 bp, Synthetic construct
  source 1..24: mol_type = other DNA
caccacaggggtttgagtaagagg

SEQ ID NO: 3 - DNA, 15 bp, Synthetic construct
  source 1..15: mol_type = other DNA
ccatccataacagcc

SEQ ID NO: 4 - DNA, 14 bp, Synthetic construct
  source 1..14: mol_type = other DNA
ccatccctaacagc

SEQ ID NO: 5 - DNA, 17 bp, Synthetic construct
  source 1..17: mol_type = other DNA
gcccatccctaacagcc

SEQ ID NO: 6 - DNA, 32 bp, Synthetic construct
  source 1..32: mol_type = other DNA
  modified_base 8: mod_base = i
agaggcgncccatccataacagcctcgcctct

SEQ ID NO: 7 - DNA, 32 bp, Synthetic construct
  source 1..32: mol_type = other DNA
  modified_base 8: mod_base = i
ggagccgncccatccctaacagcctcggctcc